European Patent Application EP 4 234 700 A2, published August 30, 2023. Title: Compositions and Methods Comprising Plants with Modified Anthocyanin Content. Applicant: Benson Hill, Inc. The sequence listing filed with the application follows.

SEQUENCE LISTING (20 sequences)

SEQ ID NO: 1 - DNA, 1558 bp, Solanum lycopersicum
  source 1..1558: mol_type = genomic DNA
atgaatactcctatgtgtgcatcgttgggagttaggaaaggttcatggactgaacaagaagattctcttttaagagattgcattcaaaaatatggtgaaggaaagtggcatcttgttcctgctagagctggtattacttttgtactttttctaatttgttttaaaaaataatgtattttatatatttataaatgatttactaaattctaagttttgattttactttctaataacataatttatagttttatgatttgttttaaatcataaatttttgtaatattttatatttatttattaattttgaatgttatgtgaacatgtataggtttaaatcgatgtcgaaagagttgcagactaaggtggctaaactatctaaggccacatatcaagagaggtgactttgctccagatgaagtggatctcatcttgagacttcacaaactcttaggcaataggtaagtctatgctgcaattatttcattcaaaagtttttgatgttatatttttttttatattgtattggtcaaatatataagtagatttttaaatttgttggatttttttcctcagatatttcaattacgtcatttttctgtataatcattgaactcccataatttgttccatttaaacaatcatcgttgtctgatgtggatcaagatttgtgagggtattgtttcacaaatcatagtccaattgatagtgaaaatgtttgagaataattgtgttttactgaagtcattttgaacacattagaaaacaaatgagactagcacggtttgtcttcattccttctatcaaaattattacaactcaaacacaatcgaagacatttacaatagaaaagctgatcaaaagtgttttaaaaaaacaaattatgggtggttcaatgattcaattgaaaaatgacgtaattgaggtacctgagaaaaaaaaacctaaacatatgtgtaattatttcatttaaaagttagttattttgtataggtggtcacttattgctggtagacttccaggaaggacagcaaacgatgtgaagaactattggaatacacactttcacaagaagttaagtattattgctcctcatctacatcctcattctcgtcctcgttctcatcctcgtctacagattaagcataagagcatcgcggttactaagaatgaaataataagacctcaacctcggaacttctcaaacgttaagaagaatgattctcattggtgcaacaacaaaagtatgatcacaaacacattagacaaagatgacaaacgttgcaacgaaatcgttgtaaatatttgtgagaagccaataggagaaaatacatcgtcgatagacgatggagttgaatggtggacaaatttactggaaaattgcattgaaattgaagaagaaacagctaatacaaattttggaaaaacaccaacaatgttgttacatgaggaaatatcaccaccgttagttaatggtgaagacaactccatgcaacaaggaccaactaataattgggatgacttttcaactgatattgacttatggaatctacttaattaa

SEQ ID NO: 2 - DNA, 828 bp, Solanum lycopersicum
  source 1..828: mol_type = other DNA
atgaatactcctatgtgtgcatcgttgggagttaggaaaggttcatggactgaacaagaagattctcttttaagagattgcattcaaaaatatggtgaaggaaagtggcatcttgttcctgctagagctggtttaaatcgatgtcgaaagagttgcagactaaggtggctaaactatctaaggccacatatcaagagaggtgactttgctccagatgaagtggatctcatcttgagacttcacaaactcttaggcaataggtggtcacttattgctggtagacttccaggaaggacagcaaacgatgtgaagaactattggaatacacactttcacaagaagttaagtattattgctcctcatctacatcctcattctcgtcctcgttctcatcctcgtctacagattaagcataagagcatcgcggttactaagaatgaaataataagacctcaacctcggaacttctcaaacgttaagaagaatgattctcattggtgcaacaacaaaagtatgatcacaaacacattagacaaagatgacaaacgttgcaacgaaatcgttgtaaatatttgtgagaagccaataggagaaaatacatcgtcgatagacgatggagttgaatggtggacaaatttactggaaaattgcattgaaattgaagaagaaacagctaatacaaattttggaaaaacaccaacaatgttgttacatgaggaaatatcaccaccgttagttaatggtgaagacaactccatgcaacaaggaccaactaataattgggatgacttttcaactgatattgacttatggaatctacttaattaa

SEQ ID NO: 3 - protein, 275 aa, Solanum lycopersicum
MNTPMCASLGVRKGSWTEQEDSLLRDCIQKYGEGKWHLVPARAGLNRCRKSCRLRWLNYLRPHIKRGDFAPDEVDLILRLHKLLGNRWSLIAGRLPGRTANDVKNYWNTHFHKKLSIIAPHLHPHSRPRSHPRLQIKHKSIAVTKNEIIRPQPRNFSNVKKNDSHWCNNKSMITNTLDKDDKRCNEIVVNICEKPIGENTSSIDDGVEWWTNLLENCIEIEEETANTNFGKTPTMLLHEEISPPLVNGEDNSMQQGPTNNWDDFSTDIDLWNLLN

SEQ ID NO: 4 - DNA, 789 bp, Solanum lycopersicum
  source 1..789: mol_type = other DNA
atgaatattgccaagacattgggagtgagaaaaggttcatggactgaagatgaagatattcttttgaggaaatgtattgacaagtatggagaaggaaagtggcatcttgttccttttagagctggtctaaatagatgtcgaaagagttgtagactgaggtggttgaattatctaaggccacatatcaagagaggtgactttgctatggatgaaatagatctcattttgagacttcacaagcttctaggcaatagatggtcacttattgctgggagacttccgggaagaacagcaaacgatgtgaaaaactattggaacacacacctacacaagaagttattaataactcctcagatacaagagaataagtacaataaaaccctcaagattatcactgaaagcactatactacgaccacgaccaagacctcgacctcgaacattctcaagtgaaaataatatttcttggtgcactaacaatagtatgatcacaaacacattagacaaagatgacgaacaacgcaacaaagaaatcgcagtaaatatttgtgagaagccaacaagagaaacaccgtcatcgtctatagacgatgatggagttaaatggtggacaaatttactggaaaattggaaagaatttgaggaagaagcaacagcagtattgaactttgaggaagaaaataagttgttaccaaatttgttgtgtgaggaacataattcaacaaccatgcaacatggagaaaatgatgacttttcagttgatattgacctatggaatctatttaattag

SEQ ID NO: 5 - protein, 262 aa, Solanum lycopersicum
MNIAKTLGVRKGSWTEDEDILLRKCIDKYGEGKWHLVPFRAGLNRCRKSCRLRWLNYLRPHIKRGDFAMDEIDLILRLHKLLGNRWSLIAGRLPGRTANDVKNYWNTHLHKKLLITPQIQENKYNKTLKIITESTILRPRPRPRPRTFSSENNISWCTNNSMITNTLDKDDEQRNKEIAVNICEKPTRETPSSSIDDDGVKWWTNLLENWKEFEEEATAVLNFEEENKLLPNLLCEEHNSTTMQHGENDDFSVDIDLWNLFN

SEQ ID NO: 6 - DNA, 1196 bp, synthetic construct
  source 1..1196: mol_type = other DNA
atgaatattgccaagacattgggagtgagaaaaggttcatggactgaagatgaagatattcttttgaggaaatgtattgacaagtatggagaaggaaagtggcatcttgttccttttagagctggtaaagcgaaattaagattttagttttataaattttaaattttatgataataaataagttctaaatttatgtagatattaagtaataatttgttaatgcaaaaataatatttaggcaaaatctattagattatactaaatttcctttttaagaaaagagaaacttaaccttttgttgtgatagtggcgtcccaacctataactctagcatgaatagcatttcatgcctccttttttattaccgagtcataaatcaatttcgttaggagtttacaaattaatatacacatatatttagttaaatttttttagttcatatataacatctaccaaaaaaattactggattcgttcaatccacaaatccccacttactattatttcatgtgaatatatgcaggtctaaatagatgtcgaaagagttgtagactgaggtggttgaattatctaaggccacatatcaagagaggtgactttgctctggatgaaatagatctcattttgagacttcacaagcttctaggcaataggtggtcacttattgctgggagacttcctggaagaacagcaaacgatgtgaaaaactattggaacacacacctacacaagaagttattaataactcctcctcagatacaagagaataagtacaataataccctcaagattatcactgaaagcactatactacgaccacgaccaagaccaggacctcaacctcgaaccttctcaagtgaaaataatatttcttggtgcactaacaatagtatgatcacaaacacattagacaaagatgacgaacaacacaacaaagaaatcgcagtaaatatttgtgagaagccaacaaaaaaaacaccgtcatcgtctatagacgatgatggagttcaatggtggacaaatttactggaaaattggaaagaatttgaggaagaagcaacagcagtattgaactttgaggaagaaaataagttgttgccaaatttgttgtatgaggaacataattcaacaaccatgcaacatggagaaaatgatgacttttcagttgatattgacctatggaatctatttaattag

SEQ ID NO: 7 - DNA, 1344 bp, synthetic construct
  source 1..1344: mol_type = other DNA
atgaatattgccaagacattgggagtgagaaaaggttcatggactgaagatgaagatattcttttgaggaaatgtattgacaagtatggagaaggaaagtggcatcttgttccttttagagctggtaaagcgaaattaagattttagttttataaattttaaattttatgataataaataagttctaaatttatgtagatattaagtaataatttgttaatgcaaaaataatatttaggcaaaatctattagattatactaaatttcctttttaagaaaagagaaacttaaccttttgttgtgatagtggcgtcccaacctataactctagcatgaatagcatttcatgcctccttttttattaccgagtcataaatcaatttcgttaggagtttacaaattaatatacacatatatttagttaaatttttttagttcatatataacatctaccaaaaaaattactggattcgttcaatccacaaatccccacttactattatttcatgtgaatatatgcaggtctaaatagatgtcgaaagagttgtagactgaggtggttgaattatctaaggccacatatcaagagaggtgactttgctctggatgaaatagatctcattttgagacttcacaagcttctaggcaataggcaagttaaaaaatatttaaaaattattgtacatatatatattcacgaaaagtaatttttgacatataaatttacgtacatactagtctctcgaatatattatagtaagttatctttgatgccatatttttatatttttttggtttagatggtcacttattgctgggagacttcctggaagaacagcaaacgatgtgaaaaactattggaacacacacctacacaagaagttattaataactcctcctcagatacaagagaataagtacaataataccctcaagattatcactgaaagcactatactacgaccacgaccaagaccaggacctcaacctcgaaccttctcaagtgaaaataatatttcttggtgcactaacaatagtatgatcacaaacacattagacaaagatgacgaacaacacaacaaagaaatcgcagtaaatatttgtgagaagccaacaaaaaaaacaccgtcatcgtctatagacgatgatggagttcaatggtggacaaatttactggaaaattggaaagaatttgaggaagaagcaacagcagtattgaactttgaggaagaaaataagttgttgccaaatttgttgtatgaggaacataattcaacaaccatgcaacatggagaaaatgatgacttttcagttgatattgacctatggaatctatttaattag

SEQ ID NO: 8 - RNA, 24 nt, synthetic construct
  source 1..24: mol_type = other RNA
acgaaatttttgatttgcctattg

SEQ ID NO: 9 - RNA, 24 nt, synthetic construct
  source 1..24: mol_type = other RNA
tatttttttggtttagatggtcac

SEQ ID NO: 10 - RNA, 24 nt, synthetic construct
  source 1..24: mol_type = other RNA
atgccatatttttatatttttttg

SEQ ID NO: 11 - RNA, 24 nt, synthetic construct
  source 1..24: mol_type = other RNA
aatattttttaacgaaatttttga

SEQ ID NO: 12 - RNA, 24 nt, synthetic construct
  source 1..24: mol_type = other RNA
atccagagcaaagtcacctctctt

SEQ ID NO: 13 - RNA, 24 nt, synthetic construct
  source 1..24: mol_type = other RNA
gttaaaaaatatttaaaaattatt

SEQ ID NO: 14 - RNA, 24 nt, synthetic construct
  source 1..24: mol_type = other RNA
tatgtcaaaaattacttttcgtga

SEQ ID NO: 15 - RNA, 24 nt, synthetic construct
  source 1..24: mol_type = other RNA
cgtacatactagtctctcgaatat

SEQ ID NO: 16 - RNA, 24 nt, synthetic construct
  source 1..24: mol_type = other RNA
taggcaataggcaaatcaaaaatt

SEQ ID NO: 17 - DNA, 953 bp, Solanum lycopersicum
  source 1..953: mol_type = genomic DNA
atggcagattggaatagatcaagcacatcagataatgcctcagtggtctcacctggtaattaacaattcttttttattttatcgcaagagcttttaattattcttttcgttcacttttattgatctattttggacatctcatgctccttaccaaaaatttcttttgatataagggtcctacagtacatattaattgatatttgatattatgttttgaaagaagatttgagaaataaataactaatgagctaagggtaaacatgaaataaaatatttgtctttttttcatgttaaaaagtaacgagtaaaaatgaacggatacttttatatttgcttataaatatattccttaaaggaatttggagaacattatgatatgattatctgcgtctaaccatatactctaataatgccataagtaaacaaatatttatccttttggctacttccaaaatacatgttcatttatgaaatcattttttttaataataagttagttagtcggaatttagaatttaaaatttatgtatttttatacatcaagttaatatattacactacttataagttcacaattaaatattcaattttgttaataattttcttaatatatttataagtctaaataaaagttattgagttcacgtgaattcattatagattcgacccgagtggttgcattagagactaccaacgaagaaacctctaaacttgaattttcagaagatgaagaaatgctcattgctaaaatgttcagcttggttagagagaggtacgtttaatatttttttaaaaaaattcttgaattttgtgtattaattatttaaggtttaatataaaattgtcatggtgtaattttaattaggtggtcattaattgctggaagaatcccaggaagaaatgctgatgagattgaaaaatattggaaatcaaaatactccaaaagccagtaa

SEQ ID NO: 18 - DNA, 255 bp, Solanum lycopersicum
  source 1..255: mol_type = other DNA
atggcagattggaatagatcaagcacatcagataatgcctcagtggtctcacctgattcgacccgagtggttgcattagagactaccaacgaagaaacctctaaacttgaattttcagaagatgaagaaatgctcattgctaaaatgttcagcttggttagagagaggtggtcattaattgctggaagaatcccaggaagaaatgctgatgagattgaaaaatattggaaatcaaaatactccaaaagccagtaa

SEQ ID NO: 19 - protein, 84 aa, Solanum lycopersicum
MADWNRSSTSDNASVVSPDSTRVVALETTNEETSKLEFSEDEEMLIAKMFSLVRERWSLIAGRIPGRNADEIEKYWKSKYSKSQ

SEQ ID NO: 20 - DNA, 1981 bp, synthetic construct
  source 1..1981: mol_type = other DNA
aaatagataataattcatgcattcaatacaagaaaatatcttaataaaaagttttaaaacgggttgaaattggagattgtattaggctcaatttagaattcttttcaaatgggctaagctttaattggttgagattgaacgtaattcaaattattctgagcccaaacccttaaaattctaggcgggttatctttgtttgaattcatttttgacatccctaatgatattgttcacgtaattaagttttgtggaagtgagagagtccaattttgataagaaaagagtcagaaaacgtaatattttaaaagtctaaatctttctacaaataagagcaaatttatttattttttaatccaataaatattaatggaggacaaattcaattcacttggttgtaaaataaacttaaaccaataaccaaagaactaataaatcctgaagtggaattattaaggataaatgtacatagacaatgaagaaataataggttcgatgaattaataataattaaggatgttacaatcatcatgtgccaagtatatacacaatattctatgggatttataatttcgttacttcacttaacttttgcgtaaataaaacgaattatctgatattttataataaaacagttaattaagaaccatcatttttaacaacatagatatattatttctaatagtttaatgatacttttaaatcttttaaattttatgtttcttttagaaaataaaaattcaaaaaattaaatatatttacaaaaactacaatcaaacacaacttcatatattaaaagcaaaatatattttgaaaatttcaagtgtcctaacaaataagacaagaggaaaatgtacgatgagagacataaagagaactaataattgaggagtcctataatatataataaagtttattagtaaacttaattattaaggactcctaaaatatatgataggagaaaatgaatggtgagagatattggaaaacttaataattaaggattttaaaatatatggtaaaagataggcaaagtatccattatccccttttaacttgaagtctactaggcgcatgtgaaagttgattttttgtcacgtcatatagctataacgtaaaaaaagaaagtaaaatttttaattttttttaatatatgacatattttaaacgaaatataggacaaaatgtaaatgaatagtaaaggaaacaaagattaatacttactttgtaagaatttaagataaatttaaaatttaatagatcaactttacgtctagaaagacccatatctagaaggaatttcacgaaatcggcccttattcaaaaataacttttaaataatgaattttaaattttaagaaataatatccaatgaataaatgacatgtagcattttacctaaatatttcaactattttaatccaatattaatttgttttattcccaacaatagaaagtcttgtgcagacatttaatctgacttttccagtactaaatattaattttctgaagattttcgggtttagtccacaagttttagtgagaagttttgctcaaaattttaggtgagaaggtttgatatttatcttttgttaaattaatttatctaggtgactattatttatttaagtagaaattcatatcattacttttgccaacttgtagtcataataggagtaggtgtatatgatgaaggaataaacaagttcagtgaagtgattaaaataaaatataatttaggtgtacatcaaataaaaaccttaaagtttagaaaggcaccgaataattttgcatagaagatattagtaaatttataaaaataaaagaaatgtagttgtcaagttgtcttcttttttttggataaaaatagcagttggcttatgtcattcttttacaacctccatgccacttgtccaattgttgacacttaactaattagtttgattcatgtatgaatactaaataattttttaggactgactca